European Patent Application EP 4 151 652 A1, published March 22, 2023. Title: ANTI-CD73 ANTIBODY AND USE THEREOF. Applicant: BIOTHEUS INC. The sequence listing filed with the application follows.

SEQUENCE LISTING (17 sequences)

SEQ ID NO: 1 - protein, 117 aa, Artificial sequence
  13D12 VH
DVKLQESGPAMVKPSQSLSLTCTVTGYSITSGYDWHWIRLFPGNKLEWMGYISYSGYTDYSPSLKSRISITHDTSKNHFFLKLHSVTTEDTATYYCTRGDHSYAMDYWGQGTSVTVS

SEQ ID NO: 2 - protein, 107 aa, Artificial sequence
  13D12 VL
DIVMTQSHKFMSTSVGDRVSITCKASQAVGTAVAWYQQKPGQSPKLLIYWASSRHTGVPDRFTGSRSGTDFTLTISSVQSEDLADYFCQQYSSYPLTFGGGTNLEIK

SEQ ID NO: 3 - protein, 8 aa, Artificial sequence
  13D12 HCDR1
GYSITSGY

SEQ ID NO: 4 - protein, 5 aa, Artificial sequence
  13D12 HCDR2
SYSGY

SEQ ID NO: 5 - protein, 9 aa, Artificial sequence
  13D12 HCDR3
GDHSYAMDY

SEQ ID NO: 6 - protein, 11 aa, Artificial sequence
  13D12 LCDR1
KASQAVGTAVA

SEQ ID NO: 7 - protein, 7 aa, Artificial sequence
  13D12 LCDR2
WASSRHT

SEQ ID NO: 8 - protein, 9 aa, Artificial sequence
  13D12 LCDR3
QQYSSYPLT

SEQ ID NO: 9 - protein, 118 aa, Artificial sequence
  7002-01 VH
QVQLQESGPGLVKPSQTLSLTCTVSGYSITSGYDWHWIRQHPGKGLEWMGYISYSGYTDYNPSLKSRITISHDTSKNQFSLKLSSVTAADTAVYYCTRGDHSYAMDYWGQGTLVTVSS

SEQ ID NO: 10 - protein, 107 aa, Artificial sequence
  7002-01 VL
AIQMTQSHSSLSASVGDRVTITCKASQAVGTAVAWYQQKPGKSPKLLIYWASSRHTGVPSRFSGSRSGTDFTLTISSLQPEDFATYFCQQYSSYPLTFGGGTKVEIK

SEQ ID NO: 11 - DNA, 351 bp, Artificial sequence
  13D12 VH nucleic acid sequence
gatgtgaagctgcaggagagcggaccagctatggtgaagcctagccagagcctgagcctgacttgcaccgtgaccggctacagcatcaccagcggctacgattggcattggatcagactgttcccaggcaacaagctcgagtggatgggctacatcagctacagcggctacaccgactacagccctagcctgaagagccggatcagcatcacccacgacaccagcaagaaccacttcttcctgaagctgcacagcgtgacaaccgaggacaccgccacctactattgcaccagaggcgaccacagctacgccatggactattggggccagggaacaagcgtgacagtgtct

SEQ ID NO: 12 - DNA, 321 bp, Artificial sequence
  13D12 VL nucleic acid sequence
gacatcgtgatgacccagagccacaagttcatgagcaccagcgtgggagacagagtgtccatcacttgcaaggcctctcaggccgtgggaacagccgttgcttggtaccagcagaagcccggacagagccccaagctgctgatctattgggccagctctagacacacaggagtgccagacagattcaccggcagcagaagcggaaccgacttcaccctgaccatcagcagcgtgcagagcgaagacctggccgactacttctgccagcagtacagcagctaccccctgacatttggcggcggcaccaacctggagatcaag

SEQ ID NO: 13 - DNA, 354 bp, Artificial sequence
  7002-01 VH nucleic acid sequence
caggtccaactccaagagagcggccccggcctcgtcaaacccagccaaacactctccctcacctgcacagtcagcggctacagcatcacaagcggatacgactggcactggatcagacaacaccccggcaaaggcctggagtggatgggctatatcagctacagcggctacaccgactacaacccaagcctgaaaagcagaatcacaatcagccacgacaccagcaagaaccagttcagcctcaagctgagcagcgtgaccgccgcagacaccgccgtctactattgcaccagaggcgaccactcctacgccatggactactggggccagggcaccctcgtgaccgtgtccagc

SEQ ID NO: 14 - DNA, 321 bp, Artificial sequence
  7002-01 VL nucleic acid sequence
gctattcaaatgacccagtcccattcctccctgtccgcctccgtgggcgaccgagtgaccattacctgtaaagccagccaagccgtcggaaccgccgtcgcatggtaccaacaaaaacccggcaaaagccccaaactcctcatctactgggccagtagcagacacaccggcgtgcccagcagattcagcggaagcagatccggcaccgacttcaccctgaccatcagcagcctgcaacccgaggacttcgccacctacttctgtcagcagtacagcagctaccccctcaccttcggaggcggcaccaaggtggagatcaaa

SEQ ID NO: 15 - protein, 330 aa, Artificial sequence
  Human IgG1-TM heavy chain constant region
ASTKGPSVFPLAPSSKSTSGGTAALGCLVKDYFPEPVTVSWNSGALTSGVHTFPAVLQSSGLYSLSSVVTVPSSSLGTQTYICNVNHKPSNTKVDKKVEPKSCDKTHTCPPCPAPEFEGGPSVFLFPPKPKDTLMISRTPEVTCVVVDVSHEDPEVKFNWYVDGVEVHNAKTKPREEQYNSTYRVVSVLTVLHQDWLNGKEYKCKVSNKALPASIEKTISKAKGQPREPQVYTLPPSREEMTKNQVSLTCLVKGFYPSDIAVEWESNGQPENNYKTTPPVLDSDGSFFLYSKLTVDKSRWQQGNVFSCSVMHEALHNHYTQKSLSLSPGK

SEQ ID NO: 16 - protein, 107 aa, Artificial sequence [sequence omitted]

SEQ ID NO: 17 - protein, 574 aa, Artificial sequence
  Human CD73
MCPRAARAPATLLLALGAVLWPAAGAWELTILHTNDVHSRLEQTSEDSSKCVNASRCMGGVARLFTKVQQIRRAEPNVLLLDAGDQYQGTIWFTVYKGAEVAHFMNALRYDAMALGNHEFDNGVEGLIEPLLKEAKFPILSANIKAKGPLASQISGLYLPYKVLPVGDEVVGIVGYTSKETPFLSNPGTNLVFEDEITALQPEVDKLKTLNVNKIIALGHSGFEMDKLIAQKVRGVDVVVGGHSNTFLYTGNPPSKEVPAGKYPFIVTSDDGRKVPVVQAYAFGKYLGYLKIEFDERGNVISSHGNPILLNSSIPEDPSIKADINKWRIKLDNYSTQELGKTIVYLDGSSQSCRFRECNMGNLICDAMINNNLRHTDEMFWNHVSMCILNGGGIRSPIDERNNGTITWENLAAVLPFGGTFDLVQLKGSTLKKAFEHSVHRYGQSTGEFLQVGGIHVVYDLSRKPGDRVVKLDVLCTKCRVPSYDPLKMDEVYKVILPNFLANGGDGFQMIKDELLRHDSGDQDINVVSTYISKMKVIYPAVEGRIKFSTGSHCHGSFSLIFLSLWAVIFVLYQ